European Patent Specification EP 4 426 865 B1, published April 1, 2026. Title: COMPOSITIONS AND METHODS FOR DETECTION OF MALARIA. Applicant: ROCHE MOLECULAR SYSTEMS, INC. The sequence listing filed with the application follows.

SEQUENCE LISTING (39 sequences)

SEQ ID NO: 1 - DNA, 27 bp, synthetic construct
  source 1..27: mol_type = other DNA; note = Description of Artificial Sequence: Synthetic primer
  modified_base 27: mod_base = OTHER; note = t-Butyl Benzyl-deoxycytidine
tgcgaaagcatttgcctaaaatacttc

SEQ ID NO: 2 - DNA, 27 bp, synthetic construct
  source 1..27: mol_type = other DNA; note = Description of Artificial Sequence: Synthetic primer
cagaacccaaagactttgatttctcat

SEQ ID NO: 3 - DNA, 31 bp, synthetic construct
  source 1..31: mol_type = other DNA; note = Description of Artificial Sequence: Synthetic probe
  modified_base 31: mod_base = OTHER; note = guanosine 3' C3 Spacer
cgtaatcttaaccataaactatgccgactag

SEQ ID NO: 4 - DNA, 27 bp, synthetic construct
  source 1..27: mol_type = other DNA; note = Description of Artificial Sequence: Synthetic primer
tgcgaaagcatttgcctaaaatacttc

SEQ ID NO: 5 - DNA, 19 bp, synthetic construct
  source 1..19: mol_type = other DNA; note = Description of Artificial Sequence: Synthetic primer
aaagttaagggagtgaaga

SEQ ID NO: 6 - DNA, 22 bp, synthetic construct
  source 1..22: mol_type = other DNA; note = Description of Artificial Sequence: Synthetic primer
aagactttgatttctcataagg

SEQ ID NO: 7 - DNA, 25 bp, synthetic construct
  source 1..25: mol_type = other DNA; note = Description of Artificial Sequence: Synthetic primer
acaactgcgaaagcatttgcctaaa

SEQ ID NO: 8 - DNA, 25 bp, synthetic construct
  source 1..25: mol_type = other DNA; note = Description of Artificial Sequence: Synthetic primer
  modified_base 25: mod_base = OTHER; note = t-Butyl Benzyl-deoxyadenosine
acaactgcgaaagcatttgcctaaa

SEQ ID NO: 9 - DNA, 30 bp, synthetic construct
  source 1..30: mol_type = other DNA; note = Description of Artificial Sequence: Synthetic primer
aactgcgaaagcatttgtctaaaatacttc

SEQ ID NO: 10 - DNA, 26 bp, synthetic construct
  source 1..26: mol_type = other DNA; note = Description of Artificial Sequence: Synthetic primer
actgcgaaagcatttgcctaaaatac

SEQ ID NO: 11 - DNA, 26 bp, synthetic construct
  source 1..26: mol_type = other DNA; note = Description of Artificial Sequence: Synthetic primer
  modified_base 26: mod_base = OTHER; note = t-Butyl Benzyl-deoxycytidine
actgcgaaagcatttgcctaaaatac

SEQ ID NO: 12 - DNA, 27 bp, synthetic construct
  source 1..27: mol_type = other DNA; note = Description of Artificial Sequence: Synthetic primer
cataaggtactgaaggaagcaatctaa

SEQ ID NO: 13 - DNA, 22 bp, synthetic construct
  source 1..22: mol_type = other DNA; note = Description of Artificial Sequence: Synthetic primer
  modified_base 22: mod_base = OTHER; note = t-Butyl Benzyl-deoxyadenosine
gacccgagaggctttgaactaa

SEQ ID NO: 14 - DNA, 29 bp, synthetic construct
  source 1..29: mol_type = other DNA; note = Description of Artificial Sequence: Synthetic primer
gatcctgagagatctttcgaaaataacca

SEQ ID NO: 15 - DNA, 28 bp, synthetic construct
  source 1..28: mol_type = other DNA; note = Description of Artificial Sequence: Synthetic probe; note = Description of Combined DNA/RNA Molecule: Synthetic probe
  modified_base 9: mod_base = OTHER; note = 5-Propynyl-2-deoxycytidine
  modified_base 10: mod_base = OTHER; note = 5-Propynyl-2-deoxyuridine
  modified_base 13: mod_base = OTHER; note = 5-Propynyl-2-deoxyuridine
  modified_base 14: mod_base = OTHER; note = 5-Propynyl-2-deoxycytidine
  modified_base 21: mod_base = OTHER; note = 5-Propynyl-2-deoxycytidine
  modified_base 22: mod_base = OTHER; note = 5-Propynyl-2-deoxycytidine
  modified_base 23: mod_base = OTHER; note = 5-Propynyl-2-deoxyuridine
  modified_base 28: mod_base = OTHER; note = guanosine 3' C3 Spacer
gcgaaagactaatcgaaaagcctattag

SEQ ID NO: 16 - DNA, 22 bp, synthetic construct
  source 1..22: mol_type = other DNA; note = Description of Artificial Sequence: Synthetic primer
gacccgagaggctttgaactaa

SEQ ID NO: 17 - DNA, 29 bp, synthetic construct
  source 1..29: mol_type = other DNA; note = Description of Artificial Sequence: Synthetic primer
  modified_base 29: mod_base = OTHER; note = t-Butyl Benzyl-deoxyadenosine
gatcctgagagatctttcgaaaataacca

SEQ ID NO: 18 - DNA, 19 bp, synthetic construct
  source 1..19: mol_type = other DNA; note = Description of Artificial Sequence: Synthetic primer
ggacccgagaggctttgaa

SEQ ID NO: 19 - DNA, 19 bp, synthetic construct
  source 1..19: mol_type = other DNA; note = Description of Artificial Sequence: Synthetic primer
  modified_base 19: mod_base = OTHER; note = t-Butyl Benzyl-deoxyadenosine
ggacccgagaggctttgaa

SEQ ID NO: 20 - DNA, 21 bp, synthetic construct
  source 1..21: mol_type = other DNA; note = Description of Artificial Sequence: Synthetic primer
gacccgagaggctttgaacta

SEQ ID NO: 21 - DNA, 21 bp, synthetic construct
  source 1..21: mol_type = other DNA; note = Description of Artificial Sequence: Synthetic primer
  modified_base 21: mod_base = OTHER; note = t-Butyl Benzyl-deoxyadenosine
gacccgagaggctttgaacta

SEQ ID NO: 22 - DNA, 30 bp, synthetic construct
  source 1..30: mol_type = other DNA; note = Description of Artificial Sequence: Synthetic primer
cctgagagatctttcgaaaataaccagcta

SEQ ID NO: 23 - DNA, 30 bp, synthetic construct; identical to SEQ ID NO: 22
  source 1..30: mol_type = other DNA; note = Description of Artificial Sequence: Synthetic primer
  modified_base 30: mod_base = OTHER; note = t-Butyl Benzyl-deoxyadenosine

SEQ ID NO: 24 - DNA, 28 bp, synthetic construct
  source 1..28: mol_type = other DNA; note = Description of Artificial Sequence: Synthetic probe; note = Description of Combined DNA/RNA Molecule: Synthetic probe
  modified_base 9: mod_base = OTHER; note = 5-Propynyl-2-deoxyuridine
  modified_base 10: mod_base = OTHER; note = 5-Propynyl-2-deoxycytidine
  modified_base 21: mod_base = OTHER; note = 5-Propynyl-2-deoxycytidine
  modified_base 22: mod_base = OTHER; note = 5-Propynyl-2-deoxycytidine
  modified_base 23: mod_base = OTHER; note = 5-Propynyl-2-deoxyuridine
  modified_base 28: mod_base = OTHER; note = guanosine 3' C3 Spacer
gtgaagaatcatacgaaaagcctaatag

SEQ ID NO: 25 - DNA, 28 bp, synthetic construct
  source 1..28: mol_type = other DNA; note = Description of Artificial Sequence: Synthetic probe; note = Description of Combined DNA/RNA Molecule: Synthetic probe
  modified_base 9: mod_base = OTHER; note = 5-Propynyl-2-deoxycytidine
  modified_base 10: mod_base = OTHER; note = 5-Propynyl-2-deoxycytidine
  modified_base 12: mod_base = OTHER; note = 5-Propynyl-2-deoxyuridine
  modified_base 21: mod_base = OTHER; note = 5-Propynyl-2-deoxycytidine
  modified_base 22: mod_base = OTHER; note = 5-Propynyl-2-deoxycytidine
  modified_base 23: mod_base = OTHER; note = 5-Propynyl-2-deoxyuridine
  modified_base 28: mod_base = OTHER; note = guanosine 3' C3 Spacer
gtgaaagaccatacgaaaagcctaatag

SEQ ID NO: 26 - DNA, 28 bp, synthetic construct
  source 1..28: mol_type = other DNA; note = Description of Artificial Sequence: Synthetic probe; note = Description of Combined DNA/RNA Molecule: Synthetic probe
  modified_base 9: mod_base = OTHER; note = 5-Propynyl-2-deoxycytidine
  modified_base 10: mod_base = OTHER; note = 5-Propynyl-2-deoxyuridine
  modified_base 21: mod_base = OTHER; note = 5-Propynyl-2-deoxycytidine
  modified_base 22: mod_base = OTHER; note = 5-Propynyl-2-deoxycytidine
  modified_base 23: mod_base = OTHER; note = 5-Propynyl-2-deoxyuridine
  modified_base 25: mod_base = OTHER; note = 5-Propynyl-2-deoxyuridine
  modified_base 26: mod_base = OTHER; note = 5-Propynyl-2-deoxyuridine
  modified_base 28: mod_base = OTHER; note = guanosine 3' C3 Spacer
gtaaaagactaattgaaaagcctattag

SEQ ID NO: 27 - DNA, 27 bp, synthetic construct
  source 1..27: mol_type = other DNA; note = Description of Artificial Sequence: Synthetic primer
tgcgaaagcatttgcctaaaatacttc

SEQ ID NO: 28 - DNA, 36 bp, synthetic construct
  source 1..36: mol_type = other DNA; note = Description of Artificial Sequence: Synthetic probe
accgtcgtaatcttaaccataaactatgccgactag

SEQ ID NO: 29 - DNA, 25 bp, synthetic construct
  source 1..25: mol_type = other DNA; note = Description of Artificial Sequence: Synthetic primer
acaactgcgaaagcatttgcctaaa

SEQ ID NO: 30 - DNA, 26 bp, synthetic construct
  source 1..26: mol_type = other DNA; note = Description of Artificial Sequence: Synthetic primer
actgcgaaagcatttgcctaaaatac

SEQ ID NO: 31 - DNA, 22 bp, synthetic construct
  source 1..22: mol_type = other DNA; note = Description of Artificial Sequence: Synthetic primer
gacccgagaggctttgaactaa

SEQ ID NO: 32 - DNA, 33 bp, synthetic construct
  source 1..33: mol_type = other DNA; note = Description of Artificial Sequence: Synthetic probe
taggggcgaaagactaatcgaaaagcctattag

SEQ ID NO: 33 - DNA, 29 bp, synthetic construct
  source 1..29: mol_type = other DNA; note = Description of Artificial Sequence: Synthetic primer
gatcctgagagatctttcgaaaataacca

SEQ ID NO: 34 - DNA, 19 bp, synthetic construct
  source 1..19: mol_type = other DNA; note = Description of Artificial Sequence: Synthetic primer
ggacccgagaggctttgaa

SEQ ID NO: 35 - DNA, 21 bp, synthetic construct
  source 1..21: mol_type = other DNA; note = Description of Artificial Sequence: Synthetic primer
gacccgagaggctttgaacta

SEQ ID NO: 36 - DNA, 30 bp, synthetic construct; identical to SEQ ID NO: 22
  source 1..30: mol_type = other DNA; note = Description of Artificial Sequence: Synthetic primer

SEQ ID NO: 37 - DNA, 33 bp, synthetic construct
  source 1..33: mol_type = other DNA; note = Description of Artificial Sequence: Synthetic probe
taggggtgaagaatcatacgaaaagcctaatag

SEQ ID NO: 38 - DNA, 33 bp, synthetic construct
  source 1..33: mol_type = other DNA; note = Description of Artificial Sequence: Synthetic probe
taggggtgaaagaccatacgaaaagcctaatag

SEQ ID NO: 39 - DNA, 33 bp, synthetic construct
  source 1..33: mol_type = other DNA; note = Description of Artificial Sequence: Synthetic probe
taggggtaaaagactaattgaaaagcctattag